European Patent Specification EP 4 326 909 B1, published January 21, 2026. Title: COMPOSITION, KIT, METHOD FOR DETECTING HIV-1 AND USE THEREOF. Applicant: SANSURE BIOTECH INC. The sequence listing filed with the application follows.

SEQUENCE LISTING (11 sequences)

SEQ ID NO: 1 - DNA, 19 bp, synthetic construct
  misc_feature 1..19: note = forward primer HIV-ZF1
  source 1..19: mol_type = other DNA
cctgggagctctctggcta

SEQ ID NO: 2 - DNA, 22 bp, synthetic construct
  misc_feature 1..22: note = reverse primer HIV-ZR1
  source 1..22: mol_type = other DNA
aagcactcaaggcaagctttat

SEQ ID NO: 3 - DNA, 20 bp, synthetic construct
  misc_feature 1..20: note = detection probe HIV-ZP1
  source 1..20: mol_type = other DNA
aggcttaagcagtgggttcc

SEQ ID NO: 4 - DNA, 21 bp, synthetic construct
  misc_feature 1..21: note = forward primer Z-POL-F1
  source 1..21: mol_type = other DNA
aaatcactctttggcarcgac

SEQ ID NO: 5 - DNA, 21 bp, synthetic construct
  misc_feature 1..21: note = reverse primer Z-POL-R1
  source 1..21: mol_type = other DNA
ccccctatcatttttggtttc

SEQ ID NO: 6 - DNA, 20 bp, synthetic construct
  misc_feature 1..20: note = forward primer Z-POL-FO
  source 1..20: mol_type = other DNA
atccctctttgggacagacc

SEQ ID NO: 7 - DNA, 20 bp, synthetic construct
  misc_feature 1..20: note = detection probe Z-POL-P1
  source 1..20: mol_type = other DNA
actgtatcatctgcycctgt

SEQ ID NO: 8 - DNA, 22 bp, synthetic construct
  misc_feature 1..22: note = internal standard forward primer
  source 1..22: mol_type = other DNA
caaagaccgttgtgtccagaag

SEQ ID NO: 9 - DNA, 22 bp, synthetic construct
  misc_feature 1..22: note = internal standard reverse primer
  source 1..22: mol_type = other DNA
cgcatgtttacacttgggtttc

SEQ ID NO: 10 - DNA, 27 bp, synthetic construct
  misc_feature 1..27: note = internal standard probe
  source 1..27: mol_type = other DNA
caacgtcctgtccaccttcctcctatg

SEQ ID NO: 11 - DNA, 475 bp, papillomavirus
  source 1..475: mol_type = genomic DNA
ttgtaagtgtgaagccagaattgagctagtagtagaaagctcagcagacgaccttcgagcattccagcagctgtttctgaacaccctgtcctttgtgtgtccgtggtgaagagtttattaatgaagatattgtaaatttgcccgagaatgtcgattggagaaaaaaaggagctgtcactcccgtaaaacatcagggttcatgcggtagttgttgggcattctcggccgttgcaactgtagagggaataaataagattagaactggaaaattagtagaattatcagagcaagaacttgttgactgtgaaagacgtagccatggggcaaagaccgttgtgtccagaagaaaaacaaagacatttggataaaaagaaacgattccacaacataggaggaaggtggacaggacgttgcatagcatgttggagaagacctcgtactgaaacccaagtgtaaacatgcgatattttatact